European Patent Application EP 4 183 874 A1, published May 24, 2023. Title: TCR-T CELL FOR TUMOR-KILLING, AND PREPARATION METHOD THEREOF AND USE THEREOF. Applicant: GUANGZHOU FINELMMUNE BIOTECHNOLOGY CO., LTD. The sequence listing filed with the application follows.

SEQUENCE LISTING (6 sequences)

SEQ ID NO: 1 - DNA, 2202 bp, Artificial Sequence
atgacggtgaaaactaaggctgctaagggcaccctcacttactccaggatgaggaaatcagatccatttctggagttcttccgccagggtaatgggaaatggcacctggtgtacagatctgaggtcatcatggatctggaaagccagaacgcatgtgctgagattgttggtgtccccacccaccccacagctctgaatcgtgtcgtggaggacttcaagaataagtacgaagatgaaattcaccaccgcacagctgctgagaatgagtttgtggtgctgggtgactactcacctttaaggattaaacacagaactgaagatgaaatcacgtaccagtgtagaaatggtttttatgtgccctcccagagaccaacgttcaagcagttggtagatgacttggatcgaattctcactctcacaaccaatgagtgcattgagtgccacctgtcagcagctggccaagcccaagaagaatgtgtggacaagtgcaaactagctggtgcgatgacgacagatttggaagggagcgacatgttggtacaaaaggctgaccggcgggagttcattgacctgttgaagaatggacagtggacactgattggacggcagagccctgagctgccacaggctttctaccctgtggggcatccagttgggggcatcgccagagagtggtttttcctcctgtctgatgaggtgctcaaccctatgtattgtttatttgaatataagcccaacaagcttcgaaatggccacaaggggctttggatcttctgcagtgaagatgagcagagccgcacctgcccggccgagtacatcagtgctgagaggatcgtgtgtaagatggaggagtcgctggtgcccagcccgccgccgggggcaaaggctagactggagctattgggtagacagttggtagcatcagcactctttgcacaatggatggatgttaatctgcagggcggaagcttcgacgtggcagacagaatgttgcacagtgtgaagagcacgtgggagtcggcctccagacggacaccactgcagaaggggcagactgcctatcagcacaaggggctgcctcagctcttctgctcgtcatcctgcactcagcaccttagtcttcaagtaccattacgatctcctagttcatcctcttcctcagaagagaacagtagttctgtggtgcgtcgccagctctttcttgacgtgcttgatgaaaccaaagcattactcctagttccagcctcagtgaacatgcagtacgcactagcagtttccaagcagcggggcccaaaacgctccctagacccgctgggaagtgaggaggagggacgatccactgttcagtttcatatattaggcatgacatgtaagatttgtgaatcctataatactgctcaagctgatggagggtcctcgctgggtttcaagcggagctacaaggaacacatcccttacacacacatgaacggaggcaagaagaggccgctgatgttggcagcattgaatgggctcttggtggctcgagtctcagggcgggaagagaatcgagttgagctgctggagatctgcgagctcagccaggagaagaggagctctgtgtttgaggacagtaacgtgtacatgttgccccagtccccgccggctccccctgtcttcctcagcacctcctgtttcgacagccaagaccactcagccttcgagaaatccacagagagattgcctggtgagcctagaggtaaagagcagattgtccctccaggaaggcagcgagccaggatggagatgggcaccgagatcagccgcaagatccggagtgccattatgatatcccatattatccgagagattcgccagtttgaacaaactgcctacaaaatagagcaccaagcaaaggtagccagcagtgggacttacaacttggactttgacaacatggagcttgtggatacctttcagaccttggagcctcgtagagaggttctgccaggagccaaatgtgattataccttacaggtgcagctaaggttctgtctctgtgagaccagcctcaccaaccagttctatctggctgctccccgaggtgtctgctacggggctgaccatgacctgggccgcctgcactgtccggacatcatcatgaacccacacggcttcccattacgaatgacggtggggaagctcattgagctgctggcttag

SEQ ID NO: 2 - DNA, 2238 bp, Artificial Sequence
atggatgagaaatgcaaacaggttctcaatgtttcccagatggtatatggccctgaaggatcagatctggttttaatgcagttctatctggctgctccccgaggtgcctgctacagggctgaccatgacctgggccgcctgcacccttgtgtgatggtgattttactttgtaacctgaaacctgcaaagataaggggagtattatctcaagcaatggtcatgtgtgctgacagcaacctcactacctacagtcgcccagggcaggctactccttacgccaccactcagctcatccagtcaaactggccagtgttccgggagcagctctgtcgtcacacatgcctcttctacatggttcgggcacaggcctggagccaggaggcctcagccctcggtctaatcctggctgactcatatgaggcctcaggcaagggcaatctggccaggctcattgaagtgaatataaccacaaacctggacttcttcctatgtgtggctcaagttcaactcttacatcagttaatagtaaaagagctggagaaatacaagaacattgatgaagatcagcttcttggcaaactctcagaagaggaactgaaacaggggcccagtgctttcagcatccctctccctatccggcagaagctctgtagcagcctggatgccccccagacgagaagccaaagggtctgcaggcctcgctctatatggagagccaagtttaggttcaatttcttttagtttgctgccaagaaacctccttgtgtagcatatgataaaaagttgcagttctattccaagatagcttatgaggttggcggggcgggtaagatggcggccccgcggcgagggaaaggatcctccacagtgctctcttcagttccccttcaagttcccccccagtattttcagcacctggatcataccgacaaacgtgtggatgcttatgaccgccctgagctatcccggtacaataagatccaggccgactaccacaatctccttggagtcacagcagagctggtggattctctagaggccccttctcttccagacagtaacactattactcaggacttcaaaaccataccttctcagaatagccagatagtaaccgaaagtcccaaacagggcagcaataaaatcaagctccagagtcgcctttcagggggtgtacaccgccttgagtcacagcaagcattcaactatctcaaccaaggggtggttcagtctataacctggaagcagatgaagccacacatacaggagctttctagcctacgttactcttcaccacaagctcctgtcaaggtggaggaaacaagaaaagacttcaggtatccgcggacttctctgcacagcatccctgtgacagtgggggtgaagccggtgctgccaagagccatgcccagttccggtgggctctgtgaaatacctggagtgctcagccctcacccagcggggcctgaagacagtgtttgaaaagtaccatcagaattgatttccctctttaataaaaaatgggatagagagattcttcttaatatccttaccctaggggagatcccagatctctactctgatgatgaagttcaaaacatcataagcaatgtgaggaatgaagtcaagagcgtgaagtctaccaagctcgtgctcaagggaaccaaggcgaagagtaagaagaaaaagagcaaagataagaaaagaaccgagcctgggaggccggccggtgccagcacctttgggcttctgagacggcggcagcagcggcattcagggactccgggcaagggggcgtcgctggatgcaggctcggggaagcccccgatggactaccacgaggatgacaagcgcttcgctagtagtgatcgggccgctgtgtgtggtgagtgtgacaaaagcttcaggcagatgtcagatctggtgaaacaccacggcctggactacctccacaccaagtgcaagatcctccacacggacatcaagcccgagaacatcttgctgtgtccaagcttaatggaacccccctctcccagggaagacaggagattgctttatctgggcttccagctgatgctatttattcttctcttctgctgggcctttgaacaagaagagaaacctaccttcaccaagctcatggacatgctggagaaactcgggtgccagtgccgcggccgcggccgccgccgacgccgccgccgccgccgccgtcgcctgggcggctgcgcctactag

SEQ ID NO: 3 - DNA, 2238 bp, Artificial Sequence
atggctggacccactaatgccatcttcaaagcctttgctgtgatcattgacaaactggaagaggacataagcagctcttggcagcaacagtcttacctggactctggaatccatcctggtgccactaccacagctccttctctgagtggtaaactgctgctgaacctggcagaagccctggcaattttgcgctgtgtggctacgcccctgctcctcgccctattctgcgcacctccaattgcaactggagtcagcagtagtgccactggaccaagcactgctaattacaattcgttctcaagtctgactgcgactcatgaagataaagagaggctggacagctgtacagcatttgctctgatgtatgagggccgccgtgcggtgctggaatatctgacggccgagatcttagagccagctggcaacgcggctcgcgacaataagaagacccgcgtggcatttaataaggaacttgatcctatacagaaaccctttgtggacaagattagagaatacaaatctaagcgacaagggatagaattctggtccaatgtctgtgatgagaaaatggatttggccattgaagcttcagaggcagcagaatcaagcttcctggcaggcgaagcatcctggctgaatgaactggatgggcacaatgacacgggcttggtctttgccagtaagtcccctgttgggtcacctctagggagcgcctttgcagaggcccccagcgagatgccaggggatgaggtgaagaagtacagccgcaatgctctcctcttcaacctgtgcttcgtgtgtgatgcccaggccaagacctgcgccctcaacacgcactatgtggcaccccgccgcctgctgctgatgggcacaccgctgcagaacaagcttcccgagctctggtctcccaacatggggatgggcactagtggaccaaatagggtcctacgcagtcaacaggtacaccctaatgggcagattgtccagcttctacctttgatcagcttcgaggctctaatacccagcccaacttacagcctgtcatgtttcggaacccagggtctgcttaatctggactgcagagagtataacgcagacaaggtcatcgtggacagtggcaccacgctgctgcgcctgcccacctggagcgtcgccttctccccagatggctcctggttagcttggtctcaaggacactgcatcgtcaaactgatcatccccttgaactaccacatagttgaggtgatctttgtagagctgtttcaacttccagcaccccctcacattgatttgctcggcgcatttccttcacctagtggtcctgcctctgtagtcttgagtggccggactcaagctcagaccaggcaagctagtgttctaattgacaggcctgccccacacttcgagcgtacatcctcactgcggcatcgacaccccagtctggctttccgaaaactgtctgagggctcctctgaccaggacgggtactttaatgcgccatgggaaaaacgagttgacctctcttggcaattaatggaaatagcagaacagcttacaaacgcagagttcctcgtgggggaccttgttgtcacccaggacacttccctaccctggcccagctcctatctcactaagagccgggcctgctacaacctgacagcactggccttgggcccccagagccggctggacaccttcgattacgactggactaagaatgccgtgctcacgtaccccagccctgccacgctggggcacctccaggcggaggctgagaagctggagatctgcatggagctcatggacacatccttggacaagctctaccggaaggtgctggataaaaacatgacaattccaatagctgccaattttcccttcttggattccttctgtgctctggacaaagatcaggatggcctaattagtaaagatagcgagagcttcggggtccccaaggggaggagccagctcaaagtgtcgaaatctccgtgtgaaaagctgatcagcactagagtgaagcaaattgccaaattgtggagaaaatcaagctcacaagaaagagcaccatatgtgcaaaaagccggcctcatcgtggttagcaaaacaggagactgggtgggaaagtggacctccacctccatgccctgggcagccgcccaagtggaacttctacggcagatgaacgaacaacatgaaaaggtttatgaacaattagacgtcacagcaagggaatag

SEQ ID NO: 4 - DNA, 2229 bp, Artificial Sequence
atgcgctggtggattgtggggtccgcctggagtggggcccggatgatcgacaacagtcaccatacgcacctgcagaagtccagcttcacccctaagcagcgcagcaaggctcgtacctgttcagaaggccgggagtgtgtcaactgtggggccctgtttctgctgtgtgacaaggaggctaagggcttcgtcaccaagcacgacctgcagggtctccagagcgacctgggtggccgctcgcccaccgtgcgtgtgtcagtggtgaccaacacgccctcgggcccggtggaggcctttgactttcagcagcaggtggtgcagctagaagggctggagaatgtcactgcccggaaccttctgggcaaactcatcaacatcgctgcgcaggtcggagcggtgcgcgtagtacgggcggttggcggcgcaggaggagccggacaaagaggggaaggagaaacctcatgctggggtctccccgcggggagtatggccaagccttggctgctagttctctacttcgctctgattgtggttccgatggcccaggtcagcatcaacaatgactacagcgagttggacttgagcacggatgccggggagcgggctcggctgcccgcgcgccgccgccgcctctactggggcttcttcttgggccgcggccgcgtcaagccgggggggcgctggcgcctggccaaacctaagagcgggacgtttcaggccctgaaggtggcctccagtgtggcatctgcctacgatgagatgagtgactgcaccggcctcccactgtccatgctgaccagcccagccacacccccggcccggggccagtaccaaatcgctgccgcgttaggctatagggagcgactagacatggtgcccgataccctgcagaaacaggcggaccactgtaacaccagggaagctctggctgagagcgaccgtgcagctaagggtctgggggctggagttgaggaggaaggagatgatgaaggaggggtctctacagagacagaaaagccaaaactaaagtttaaggaaaaaaataaaaatagtgatggaggaattctgcaagcaactgggttcccatggcatgtggtggtcttagaggaggtgttcagcctgccaccgtcggtgcttaagcaagccctgaaaaagcccatcaagggcaaacagcccccccgaaaaaaagctcaaggaaaaacgcaacagaatgccgccctgggcaagcaggcgagcttctcgggcagcctggaggtcatcgaggtgtccgggctggagctggaggagctggtgccgcgcctgttcctggtggcgtccaaaagacacggggaccttctggaggtaatggcccaggcgtctcgctcaggtagcctgcttccactcgttatcgtgcccccgctgagggcgcaacccgaagaagctgtggtcatggtagaggttaaccagagcgcaaagaaacaagtcatcttgtcctcagggacagaattctccattctggtgcagtgccactacaggctccaggatgccaaagctcagaaggtgtggtgccggttcttgccggaggagctgtcgagtcagctcttctactacggaggggaaccgcagagccagaagagcacggagcagcaactcgcagccgacaccaccctctacataccgagaacggcggacaaaactctttttccaggtcatctgcacgacgcagcgctcaacctcactgacacccaagtcaagaccttgtaccagaaccgcaggaccaagtggaagcggcagacaatgagtaaatatccatctggtgagagagtacgttatcaatgtaggagcccttatgaaatgtttggggatgaagaacttaatgtccttgacaacaaaaagaggacagctctgacaaaggccgtacaatgccaggaagatgaatgtgcgttagcaaaagcattttggagaatggataggcttttaggtcatggaagaaaagaagtgtccagggttcaatggagtggccgaccactgtgcaagtttgctcatgtgcctgaacaaagggatgaaaaggtttgcatggatgtgtttaagaaatatctcgcccccaaagggcaacccggacccgctgccactaataggaaccctagaggctccagcagcagacagagcagctttgtgaaagcatcaaagcgctttgaagagtccaaagacattactccaggcccagcaacatatgagatatcccagtag

SEQ ID NO: 5 - DNA, 2433 bp, Artificial Sequence
atggcacagcctgctcaacctgctgatgaacctgcagaaagggctgatgaaccaatggaacataagaagatggatctcattgacctagaggatgagaccgttgatgccgaggtcatgaactctctagcagttactatgggcataaccatccctggtatctcttcagatgtgccagacagtgcccacaaaactactgcctcagaggcaaagtcagccagacctcatccattccaaaatatgcccggtgctacccgcccagctgctcctagaccaccatttagtactatggtcacccacgctcctcagcccctgcttcccggttccgacaggcccctgccctgtgggccccaggaggccgcatgcggcctgccatcgctgccaccaccacctgcggcccctacctcagggccgcccctgagcgccacgcagatcaaacagtacaagcagtcacagcacatgacggaggttgtgaggcactgcccccaccatgagcgctgctcagatagcgatggtcttgagaaacttcgccagcgaatacatgataaagctgtgctctggagcgggctacgtgatatgaagagctgtcagtttgtagccgtcagaggagatactggagaaaagctgacagttgctgaaaatgagtttctgctgcacccgagtgatcatgaaaatattcagacattttcagatgaatttgccagaagggctaatggaaattatgctaaaaataaagcagttggagtgatgaagtcgagccatgtatttacaattgagccaatgatttgtgaaggcggcgagccggtggagttcagatgcatcctggaggctcataatgttcccgaccgttactttgctgtctcctgggccctcaatggatgtgaaaatggtcgctgtgtgagggtcaaggaaggttacacctgcgattgctttgatgggtatcacaaaactgaaacaatgaatgtagttatggagaccaatagaatgctaagagaagagaaggagagactagaacaggatcatggagacaaagacaaaatggttgctgttgcctcacagagtagcatcatcttgtggagtgttcaggatgggggagacaagaacaaggccaacagagagtcactctatgacgtttgggagtactatctcccctacctctactcatgcatcggcatcctgcttccccagttcctgggggtgctgctgatgctgctgtacatcacccgggtggaggacatcatcatgatgaacaacttcctgggcagtgagcccatcctgatgctcacactgggatcccagcctgtcctcaagaccgacaacagaaatgctactggtcctcgtcctgctttatttgtggctgaggtttcatttgagttactggtgaagcggcaaatccttcacgtggagaagttcatcagcgtgcacgagaacggccagagcagtgctgatggtgccagtgaacgtgctgttctgctccagggcaggggcctgcaagaggaagaggagttctgcatggccccgcgcagctctcagagctcagaagaggtcatccttggcatggatgatacacaggtgcgaagttctgctactgatatattctcatacttggttgaatataatgacagtaagctcaaggacatgcgagatgaggtcctgcaacatgagctgatggtggctgaccggcgccagaagcgatgcgagctgcccagcaccatccccatcaagcagaacacccgccgcagcagctggagctctgacgaagggatcgggtgcacagaagctgtttttttattattgggaatgctccacagcatgctgacttcaccttggcaatcagaagaagagctcaaacgcagcaaagcctccatctcctcctcctcctcctcagccccagcgatgccagcacttcctcattccccaccagctctgatggcctctctcccttctcggagaccttcatccctgactccagcaagggccttggccccagggcacccgcatccccggcaccagcccaggcccagacccccacccctgctccagccccagcctcctcccaagcaccccttcggccagaggatgacattctgtaccagtggcggcagcggcggaagcttgaacaggctcagggaagcaagggtgacagagcttgggtgccgcctccaagttgtggttcctggtataaatttacccgtcaatcatctgacctatttcttcacggcagttctcattagtggtcacatcaaggccaagcacaggaatgagaggccacacgcatgtgagttctgcagccacgccttcacccaaaaggccgacctagtggaagggttacatgatggacacttctacaccctgaagcgaatcctgtgtcacgagcagcaggaccggatgactggcatcttccattttgccattatcttcatgttaatactttaa

SEQ ID NO: 6 - DNA, 2358 bp, Artificial Sequence
atgaggctccatccagtcccagtcccagcagattggatgaaacgcatggaggtgaatgagacccagtacaatgagatgacttccttctgcgtctgcacaggccctgggcaccagcaggctatgctttcacccacctcagcctgcaggagtttcttgctgccctgcaccagaggtggccgggggcgcccaagggggcagcctcctatgcccccaaagccttccatcaggccccggccagggagcatgtccctcgagagaccccccagggtgcctccgagatctgcctcacagaggcctccgaccagggagaccttccatccctttgctgatgatgtggaggacacctatgacgacgagactgaggactcaagcctgcaggagaaattcttcacgttccctaaggccccttctaagctgacagtggggggggccatggggccaaagtcaggaaaaggaaaagggagacaagaattcagccaccccgaaacagaagccattgcctcccttgtttaccttgggtccacctccaccaaaacccaacagaccaccaaatgtaccaagaacaaccagttccaggccctgctgcagtatgtggaccccgtgagcgcccagcacgccaagctgtcgctgagacctgccagcccttcagcaccactgcaggataacggaactcaaggcttaattaacggggcactaaacaaaacagaaaggatccgagatctaagtggcaatctttgggagcattccagtggggatggagaagaactagaaagacttaccgaagttagcatgatagtaaattcacataagccccaaaagaatttggattctatacaagttaccaaagatctcacatccttaaagttttttcagaaaaaggaaactaagagaggtttggatttcacagattctcaagaaaatgaagaaaaagcttcctgtggcacagagggatttcggaatgccaaggagggcacaggcatcgcagcacagacagcaggcatagccctgtggccttcagacagcgccgcaccgcggctgggctcctcggagatcatgcatgccccgcggtccagggacagggccactgaattttttgaagatgacgccacattaaccccttcattttgtttggaagatggaccaaagcgatacactaacagtgaatgtgcaagtaaagatgttctggtgaagaacctcagggctattgatgtgaaacttaactctgataatatggagcaagagaggaatgctcgctaccgaacccccagaatcttggagcccacagccttccaggaacccccacccccccctttgtgggaaaagcctcccttgggaagcagtagttgtatgctcagtcctcccctgggaagaacaacaacacctaccaccacccggggtctctgggcaataagtgagagagagcgatctatgaaagcaatactatcatttgcaaaaataaagcagttaaacatttcacacttactagtacctccgggattagccaaaccagctcatctttatgacaaagggtgtgtagaagagaggatatgtcacctccaacgtgaaattgcgtggcttgtacagcaactagatgacgttcatcagtttggttcagtgaccaacataccagcaaaggatgcaccaccagtggagaaaatagacaccatgctggtcttggaacttgggcttgccttcaacttgaatccagctctgaccataattggcaagtatttctacaagaggcgaccattggccagccagcttccccattgcccctctgtatctcccagtacccagccttggacacaccctggccagagccagctgtttgacttcacttgtgatgacggaaatgatgacaatagttactccccactttctcgctgtcctactgaatgtacttgcaaacacgatgaaaacctgtatggtcccattgtgaaacgtatttcattttttgatttcttcaagcataagtatcaacacctcaaagctcttaaatgcttatctctggtacccgcagtcatgggacaactcaaattcaatacgtcggaggaaggagccagcatattccagtccaaagagtcctcgtcagagcttagctgtgacatctctgtggatgataagtacatatacatgagacggcccaatccagttagtccttatccaatctcttcacacacttcagatatctatggaagcaccagcttcaaccatcacccctacccccacaaccactacatggcggatttgcaccctgctgcaggccaccagatgaacgggaagtggggtggctgtagcgaggacatcgagtttggtgagatggtgtctcgggagttcgccgacgcccgggagaactga